European Patent Application EP 4 534 103 A1, published April 9, 2025. Title: PHARMACEUTICAL COMPOSITION OF RECOMBINANT ANTI-HUMAN CLDN18.2 MONOCLONAL ANTIBODY-MMAE CONJUGATE. Applicant: CSPC Megalith Biopharmaceutical Co., Ltd. The sequence listing filed with the application follows.

SEQUENCE LISTING (19 sequences)

SEQ ID NO: 1 - protein, 8 aa, synthetic construct
GFTFSSYA

SEQ ID NO: 2 - protein, 8 aa, synthetic construct
LSGSGRST

SEQ ID NO: 3 - protein, 13 aa, synthetic construct
AKSLSYYHYYFDY

SEQ ID NO: 4 - protein, 6 aa, synthetic construct
QDISNY

SEQ ID NO: 5 - skipped

SEQ ID NO: 6 - protein, 9 aa, synthetic construct
QQVKTYPLT

SEQ ID NO: 7 - protein, 120 aa, synthetic construct
EVQLSESGGALVQPGESLRLSCAASGFTFSSYAMTWVRQAPGKGLEWVSSLSGSGRSTYYAASIKGRFTISRDNSKNTLYLQMSSLRAEDTAIYYCAKSLSYYHYYFDYWGQGTLVTVSS

SEQ ID NO: 8 - protein, 107 aa, synthetic construct
DIQLTQSPSFLSASVGDRVPITCRASQDISNYLAWYQQKPGKAPKLLIYSASTLQSGVPSRFSGSGSGTEFTLTISSLQPEDFASYHCQQVKTYPLTFGGGTKVEIK

SEQ ID NO: 9 - protein, 450 aa, synthetic construct
EVQLSESGGALVQPGESLRLSCAASGFTFSSYAMTWVRQAPGKGLEWVSSLSGSGRSTYYAASIKGRFTISRDNSKNTLYLQMSSLRAEDTAIYYCAKSLSYYHYYFDYWGQGTLVTVSSASTKGPSVFPLAPSSKSTSGGTAALGCLVKDYFPEPVTVSWNSGALTSGVHTFPAVLQSSGLYSLSSVVTVPSSSLGTQTYICNVNHKPSNTKVDKKVEPKSCDKTHTCPPCPAPELLGGPSVFLFPPKPKDTLMISRTPEVTCVVVDVSHEDPEVKFNWYVDGVEVHNAKTKPREEQYNSTYRVVSVLTVLHQDWLNGKEYKCKVSNKALPAPIEKTISKAKGQPREPQVYTLPPSRDELTKNQVSLTCLVKGFYPSDIAVEWESNGQPENNYKTTPPVLDSDGSFFLYSKLTVDKSRWQQGNVFSCSVMHEALHNHYTQKSLSLSPGK

SEQ ID NO: 10 - protein, 214 aa, synthetic construct
DIQLTQSPSFLSASVGDRVPITCRASQDISNYLAWYQQKPGKAPKLLIYSASTLQSGVPSRFSGSGSGTEFTLTISSLQPEDFASYHCQQVKTYPLTFGGGTKVEIKRTVAAPSVFIFPPSDEQLKSGTASVVCLLNNFYPREAKVQWKVDNALQSGNSQESVTEQDSKDSTYSLSSTLTLSKADYEKHKVYACEVTHQGLSSPVTKSFNRGEC

SEQ ID NO: 11 - protein, 25 aa, synthetic construct
EVQLSESGGALVQPGESLRLSCAAS

SEQ ID NO: 12 - protein, 17 aa, synthetic construct
MTWVRQAPGKGLEWVSS

SEQ ID NO: 13 - protein, 38 aa, synthetic construct
YYAASIKGRFTISRDNSKNTLYLQMSSLRAEDTAIYYC

SEQ ID NO: 14 - protein, 11 aa, synthetic construct
WGQGTLVTVSS

SEQ ID NO: 15 - protein, 26 aa, synthetic construct
DIQLTQSPSFLSASVGDRVPITCRAS

SEQ ID NO: 16 - protein, 17 aa, synthetic construct
LAWYQQKPGKAPKLLIY

SEQ ID NO: 17 - protein, 36 aa, synthetic construct
TLQSGVPSRFSGSGSGTEFTLTISSLQPEDFASYHC

SEQ ID NO: 18 - protein, 10 aa, synthetic construct
FGGGTKVEIK

SEQ ID NO: 19 - protein, 331 aa, synthetic construct
DSDERVTPPAEPLDRMPDPYRPSYGRAETIVNNYIRKWQQVYSHRDGRKQQMTEEQREWLSYGCVGVTWVNSGQYPTNRLAFAFFDEDKYKNELKNGRPRSGETRAEFEGRVAKDSFDEAKGFQRARDVASVMNKALENAHDEGAYLDNLKKELANGNDALRNEDARSPFYSALRNTPSFKDRNGGNHDPSKMKAVIYSKHFWSGQDRSGSSDKRKYGDPEAFRPDRGTGLVDMSRDRNIPRSPTSPGESFVNFDYGWFGAQTEADADKTVWTHGNHYHAPNGSLGAMHVYESKFRNWSDGYSDFDRGAYVVTFVPKSWNTAPDKVTQGWP